European Patent Application EP 4 159 858 A1, published April 5, 2023. Title: RNAi AGENTS TARGETING MYELOID DIFFERENTIATION PRIMARY RESPONSE 88 AND METHOD OF USE THEREOF. Applicant: OliX Pharmaceuticals, Inc. The sequence listing filed with the application follows.

SEQUENCE LISTING (4 sequences)

SEQ ID NO: 1 - RNA, 19 nt, Artificial Sequence
  MyD88 siRNA_antisense
uggucuggaagucacauuc

SEQ ID NO: 2 - RNA, 16 nt, Artificial Sequence
  MyD88 siRNA_sense
ugugacuuccagacca

SEQ ID NO: 3 - DNA, 20 bp, Artificial Sequence
  MyD88 Forward primer
gctcatcgaaaagaggtgcc

SEQ ID NO: 4 - DNA, 20 bp, Artificial Sequence
  MyD88 Reverse primer
ggttggtgtagtcgcagaca